European Patent Application EP 4 578 872 A1, published July 2, 2025. Title: 一种抗TREM2的单域抗体及其用途. Applicant: 南京融捷康生物科技有限公司. The sequence listing filed with the application follows.

SEQUENCE LISTING (50 sequences)

SEQ ID NO: 1 - protein, 116 aa, synthetic construct
ESGGGLVQAGESLRLSCAASGRTFTNYAMGWFRQAPGKEREFVAGVSWSGSSTDYADSVKGRFTISTDNAKNTVYLQINNLKPEDTAVYICGVKYFGHSRGGYDYWGQGTQVTVSS

SEQ ID NO: 2 - protein, 110 aa, synthetic construct
ESGGGLVQPGGSLRLSCAASGFTFSGYYMSWVRQVPGKARELVAGITRGGNTYYADSVKGRFTISRDNAKNTVYLQMNNLKPEDTTVYYCNARRATTYYWGQGTQVTVSS

SEQ ID NO: 3 - protein, 112 aa, synthetic construct
ESGGGLVQPGGSLRLSCAASGFAFGNYVMHWYRQAPEKERELVAIIGSQGGTYTNYADSVKGRFTISRDNAKNMVYLQMNNLKPEDTAVYYCNVVYIGRPNWGQGTQVTVSS

SEQ ID NO: 4 - protein, 116 aa, synthetic construct
ESGGGLVQAGESLRLSCAASGRTFTDYAMGWFRQAPGKEREFVAGVSWSGSSTDYADSVKGRFTISTDNAKNTVYLQMTSLKPEDTAVYICGVKYFGHSRGGYDYWGQGTQVTVSS

SEQ ID NO: 5 - protein, 110 aa, synthetic construct
ESGGGLVQPGGSLRLSCAASGLTFSEYYMSWVRQVPGKARELVAGITRGGNTYYADSVKGRFTISRDNAKNTVYLQMNNLKPEDTTVYYCNARRATTYYWGQGTQVTVSS

SEQ ID NO: 6 - protein, 116 aa, synthetic construct
ESGGGLVQAGESLRLSCAASGRTFTNYAMGWFRQAPGKEREFVAGVSWSGSSTDYADSVKGRFTISTDNAKNTVYLQMTSLKPEDTAVYICGVKYFGHSRGGYDYWGQGTQVTVSS

SEQ ID NO: 7 - protein, 117 aa, synthetic construct
ESGGGLVQPGGSLRLSCAASGRTFSSYVMGWFRQAPGKEREFVAAISWSGGITYYGDSVKGRFTISRDNAKNTVFLQMNSLKPEDTAVYYCASGSGSYYRGWEYDYWGQGTQVTVSS

SEQ ID NO: 8 - protein, 112 aa, synthetic construct
ESGGGLVQPGGSLRLSCAASGFAFSNYVMHWYRQAPEKERELVALIGSQGGAYTNYAGSVKGRFTISRDNTKNMVYLQMNNLKPEDTAVYYCNVVYNGRPNWGQGTQVTVSS

SEQ ID NO: 9 - protein, 112 aa, synthetic construct
ESGGGLVQPGGSLRLSCAASGFAFSNYVMHWYRQAPEKERELVAIIGSQGGAYTNYAASVKGRFTISRDNAKNMVYLQMNNLKPEDTAVYYCNVVYIGRPNWGQGTQVTVSS

SEQ ID NO: 10 - DNA, 348 bp, synthetic construct
  source 1..348: mol_type = other DNA
gagtctggaggaggattggtgcaggctggggaatctctgagactctcctgtgcagcctctggacgcaccttcactaattatgccatgggctggttccgccaggctccagggaaggaacgtgagtttgtagccggtgttagctggagtggtagtagcacagactacgcagactccgtgaaaggccgattcaccatctccacagacaacgccaagaacacggtgtatctgcaaataaacaacctgaaacctgaggacacggccgtttatatctgtggagtaaaatatttcggacatagtcgcggggggtatgattattggggccaggggacccaggtcaccgtctcctca

SEQ ID NO: 11 - DNA, 330 bp, synthetic construct
  source 1..330: mol_type = other DNA
gagtctggaggaggcttggtgcagcctggggggtctctgagactctcctgtgccgcctctggattcaccttcagtggatactacatgagttgggtccgccaggtaccagggaaggcgcgcgaattggtcgcaggaattactagaggtggtaatacatactatgcagactccgtgaagggccgattcaccatctccagagacaatgccaaaaacacggtgtatctgcaaatgaacaacctgaaacctgaggacacgaccgtctattactgtaacgcccgccgagcaacgacctattactggggccaggggacccaggtcaccgtctcttca

SEQ ID NO: 12 - DNA, 336 bp, synthetic construct
  source 1..336: mol_type = other DNA
gagtctgggggaggcttggtgcagcctggggggtctctgagactctcctgtgcagcctctggattcgccttcggtaactatgtcatgcactggtaccgccaggctccagagaaggagcgcgagttggtcgcaattattggtagtcaagggggtacctacacaaactatgcagactccgtgaagggccgattcaccatctcccgagacaatgccaagaacatggtgtatctacaaatgaacaacctgaaacctgaggacacggccgtgtattactgtaatgtcgtgtacattgggcgccccaactggggccaggggacccaggtcaccgtctcctca

SEQ ID NO: 13 - DNA, 348 bp, synthetic construct
  source 1..348: mol_type = other DNA
gagtctggaggaggattggtgcaggctggggaatctctgagactctcctgtgcagcctctggacgcaccttcactgattatgccatgggctggttccgccaggctccagggaaggaacgtgagtttgtagccggtgttagctggagtggtagtagcacagactacgcagactccgtgaagggccgattcaccatctccacagacaacgccaagaacacggtgtatctgcagatgacaagcctgaaacctgaggacacggccgtttatatctgtggagtaaaatatttcggacatagtcgcggggggtatgattattggggccaggggacccaggtcaccgtctcctca

SEQ ID NO: 14 - DNA, 330 bp, synthetic construct
  source 1..330: mol_type = other DNA
gagtctggaggaggcttggtgcagcctggggggtctctgagactctcctgtgccgcctctggactcaccttcagtgaatactacatgagctgggtccgccaggtaccagggaaggcgcgcgagttggtcgcaggaatcactagaggtggtaacacatactatgcagactccgtgaagggccgattcaccatctccagagacaatgccaaaaacacggtgtatctgcaaatgaacaacctgaaacctgaggacacgaccgtctattactgtaacgcccgccgagcgacgacctattactggggccaggggacccaggtcaccgtctcctca

SEQ ID NO: 15 - DNA, 348 bp, synthetic construct
  source 1..348: mol_type = other DNA
gagtctggaggaggattggtgcaggctggggaatctctgagactctcctgtgcagcctctggacgcaccttcactaattatgccatgggctggttccgccaggctccagggaaggaacgtgagtttgtagccggtgttagctggagtggtagtagcacagactacgcagactccgtgaagggccgattcaccatctccacagacaacgccaagaacacggtgtatctgcagatgacaagcctgaaacctgaggacacggccgtttatatctgtggagtaaaatatttcggacatagtcgcggggggtatgattattggggccaggggacccaggtcaccgtctcctca

SEQ ID NO: 16 - DNA, 351 bp, synthetic construct
  source 1..351: mol_type = other DNA
gagtctgggggaggcttggtgcagcctgggggttctctgagactctcctgtgcagcctctggacgcaccttcagtagctatgttatgggctggttccgccaggctccagggaaggagcgtgagtttgtagcagctattagctggagtggtggcatcacatactatggagactccgtgaagggccgattcaccatctccagagacaacgccaagaacacggtgtttctgcaaatgaacagcctgaaacctgaggacacggccgtttattactgtgcgtcggggagtggtagttactaccgcgggtgggagtatgactactggggccaggggacccaggtcaccgtctcctca

SEQ ID NO: 17 - DNA, 336 bp, synthetic construct
  source 1..336: mol_type = other DNA
gagtctgggggaggcttggtgcagcctggggggtctctgagactctcctgtgcagcctctggattcgccttcagtaactatgtcatgcactggtaccgccaggctccagagaaggagcgcgagttggtcgcacttataggtagtcaagggggtgcctacacgaactatgcaggctccgtgaagggccgattcaccatctcccgagacaataccaagaacatggtgtatctacaaatgaacaacctgaaacctgaggacacggccgtgtattactgtaatgtcgtgtacaacgggcgccccaactggggccaggggacccaggtcaccgtctcctca

SEQ ID NO: 18 - DNA, 336 bp, synthetic construct
  source 1..336: mol_type = other DNA
gagtctgggggaggcttggtgcagcctggggggtctctgagactctcctgtgcagcctctggattcgccttcagtaactatgtcatgcactggtaccgccaggctccagagaaggagcgcgagttggtcgcaattattggtagtcaagggggtgcctacacaaactatgcagcctccgtgaagggccgattcaccatctcccgagacaatgccaagaacatggtgtatctacaaatgaacaacctgaaacctgaggacacggccgtgtattactgtaatgtcgtgtacattgggcgccccaactggggccaggggacccaggtcaccgtctcctca

SEQ ID NO: 19 - protein, 20 aa, synthetic construct
ESGGGLVQAGESLRLSCAAS

SEQ ID NO: 20 - protein, 20 aa, synthetic construct
ESGGGLVQPGGSLRLSCAAS

SEQ ID NO: 21 - protein, 17 aa, synthetic construct
MGWFRQAPGKEREFVAA

SEQ ID NO: 22 - protein, 17 aa, synthetic construct
MGWFRQAPGKEREFVAG

SEQ ID NO: 23 - protein, 17 aa, synthetic construct
MHWYRQAPEKERELVAI

SEQ ID NO: 24 - protein, 17 aa, synthetic construct
MHWYRQAPEKERELVAL

SEQ ID NO: 25 - protein, 17 aa, synthetic construct
MSWVRQVPGKARELVAG

SEQ ID NO: 26 - protein, 38 aa, synthetic construct
DYADSVKGRFTISTDNAKNTVYLQINNLKPEDTAVYIC

SEQ ID NO: 27 - protein, 38 aa, synthetic construct
DYADSVKGRFTISTDNAKNTVYLQMTSLKPEDTAVYIC

SEQ ID NO: 28 - protein, 38 aa, synthetic construct
NYADSVKGRFTISRDNAKNMVYLQMNNLKPEDTAVYYC

SEQ ID NO: 29 - protein, 38 aa, synthetic construct
NYAASVKGRFTISRDNAKNMVYLQMNNLKPEDTAVYYC

SEQ ID NO: 30 - protein, 38 aa, synthetic construct
NYAGSVKGRFTISRDNTKNMVYLQMNNLKPEDTAVYYC

SEQ ID NO: 31 - protein, 38 aa, synthetic construct
YYADSVKGRFTISRDNAKNTVYLQMNNLKPEDTTVYYC

SEQ ID NO: 32 - protein, 38 aa, synthetic construct
YYGDSVKGRFTISRDNAKNTVFLQMNSLKPEDTAVYYC

SEQ ID NO: 33 - protein, 11 aa, synthetic construct
WGQGTQVTVSS

SEQ ID NO: 34 - protein, 8 aa, synthetic construct
GFAFGNYV

SEQ ID NO: 35 - protein, 8 aa, synthetic construct
GFAFSNYV

SEQ ID NO: 36 - protein, 8 aa, synthetic construct
GFTFSGYY

SEQ ID NO: 37 - protein, 8 aa, synthetic construct
GLTFSEYY

SEQ ID NO: 38 - protein, 8 aa, synthetic construct
GRTFSSYV

SEQ ID NO: 39 - protein, 8 aa, synthetic construct
GRTFTDYA

SEQ ID NO: 40 - protein, 8 aa, synthetic construct
GRTFTNYA

SEQ ID NO: 41 - protein, 9 aa, synthetic construct
IGSQGGAYT

SEQ ID NO: 42 - protein, 9 aa, synthetic construct
IGSQGGTYT

SEQ ID NO: 43 - protein, 8 aa, synthetic construct
ISWSGGIT

SEQ ID NO: 44 - protein, 7 aa, synthetic construct
ITRGGNT

SEQ ID NO: 45 - protein, 8 aa, synthetic construct
VSWSGSST

SEQ ID NO: 46 - protein, 15 aa, synthetic construct
ASGSGSYYRGWEYDY

SEQ ID NO: 47 - protein, 14 aa, synthetic construct
GVKYFGHSRGGYDY

SEQ ID NO: 48 - protein, 9 aa, synthetic construct
NARRATTYY

SEQ ID NO: 49 - protein, 9 aa, synthetic construct
NVVYIGRPN

SEQ ID NO: 50 - protein, 9 aa, synthetic construct
NVVYNGRPN